European Patent Specification EP 3 873 488 B1, published March 19, 2025. Title: COMPOSITIONS AND METHODS FOR TREATING VIRAL INFECTIONS. Applicant: The University of Sydney The Westmead Institute for Medical Research. The sequence listing filed with the application follows.

SEQUENCE LISTING (7 sequences)

SEQ ID NO: 1 - DNA, 10901 bp, Homo sapiens
agggaggtgccagatgcagtggcagagccaaggctggggtgatataccaccctttgttctttcctgacgctgtggctgaggcagagcaaagagtaacattggtgggcttggcctgggtgcccatgaatgagggctgcccagaaggcagtgggccaggaccctgagcacagcggggtagttctctgcagccagtggttcagggaatcctggcactgggtcccaggcattcagccatccaagtcacttctcagttctcagcaacctggaggctcaccaggctcagggcatggactttaccccttgccaggggacgaggcctccaagtgctgtgtgcgtgtgcaggtgcatcctgtacacgggacaaggccaagcccctaggctgagctgggcacaggcaccctggccttgtgtggagaaggtggggtgggggtggcaggcagggctgcctggaggaggggatgctggggcccgcttacaagaaggctcattttacagacagaaagcaggcctggggggtgttgaccctgctagagttggggaaagtccaggggaacctgaacttcacccatgggcagtggacacctggggaaggaggctgagtcagacctgcggccagaagaccctcttgtggcccagttcaggaagacctgtgacccagttggcatcaagctaaggggctgcgtgcagaatggggcctgaggtaggggcagtggttagaatttgtgccagctgcagactggggtcccgcagggcaggcgtcaggtgggcatggttcaccttgctgtctgcagcatccacaagtactccacatgggccagagtctggttggagggggtgacaaagacagatggtctccttattctcccccccaatactgtggccccctcccagctgttcaaaacctcccacagcctctcacagctgtctcgcttctcatcacaccccagcagaaccgacctcctttccactgctcagttccaagcctgagccactttcctccctgccaggaacaccgttcccaaactcttcaccaaactggctccatcccgatattctaacttcagcccccacccgctaggaccccttctaccctctccccgaaatgaagaaccctaaacccgggactagcctgcaaagggacagccccggagtcaaagcctcacacttaaagacccctcgcagtggctcacgcctgtaatcccagctcctcgggaggctgatgtgggaggatctgttgagcccaggagtttgaaaccagtctgggcaaaaaagtgagacctctgtctttacaaaaaataactagctgcgcgtggtggtgcatacctgtagtcccaactacttgggaggctgaggtaggaggatctcttgaggctgggagttcaaggaggagggccactgcactccagtctgggccacagagtgagacctctcaaaaaacaaacaaaaaaacttcacacctgcctggaaacacgtttacatttgtggccaccttatgaaaactcaaatctaagcccactgaaaggcattttgcacccaagagctggaggttgctccatccgtgcgcacagggaatgccgacttgatctttgggtggggatgggaaactctggggaatgcagaggtttagaagcgcagagtccaggagaaaatttccttagaacgaagttgtggaggcaggggaaagagggggcacgccaggacctccagggcgcaccccttggcctaagagcagaagcatcccgaggtgttgtgtcccagcctttgacagtgagggaaactgaggctgagtagcgggacggccattggagacgagggtgtcgatggtgaggggcgaaggggcggggcagctgccagggggagggccggggaggggccttggaggctccctgggaacacgcagggcggtcacggcggcctgcccagggcgcagcggggtcgacctttgtgcggggcgggtccctggcagcctcggcccggactcgccgccaacgaggagccgagcgccctggagaacgcgtcggggctgagccggggtccagcagccgccgctatggacatcccgccgctggccggcaagatcgcggcgctgtcgctgagcgccctcccggtgtcctacgcgctcaaccacgtctcggcgctctcgcagtgcgtgcggagaggggccagggcggccttggggacagtgggggcgggcgggggcggggaggactggaggtgggctggagggaggatgcgcggtccgcggacctggcttctgcgagccctgcgccccagctcagctccgacccggcaggattggggtgggccagaagaacacccccctctaaccggaagtccccttcccgccgggctggaggctgggatgcggccgctcctgggatgtttgtggcctgggaagaaggaatgatgagtccccacaagccagagctttggagggtttctggggttttcccagggatgcgccctgcctaggttccaaagtcaccaagggtaaaagtattgtcccagataaggccccgggtacctgactcctgctcacacacacacacacacacacacacacacacacacaccctactccattgcctgtctcaggcctgtgactttcctcttgttcagggctggctaaccatgtccctagactcagttccccctactggttccctttcctggtccctgtctcctaaccctagatcctagccctgtgggtccagccaccggatagtgggcatctgcaagcccctcgtacttctaaacccagctcaacccaagccatggggtggagagagtcttaaccatgagcctggctccctgggtgggaatacccatctccatctcctgggatcctgggtgagccaagttcctctgggagcctcagttccctcatcagtgtaatgggcacgatcctagatctcatctcatagttacggttaaggattataaactgtgtacaaagatttgtcttggtctcatctgagtactataatgtcattgttagatggggtcaggatggaaatcttgggttctgaggggatcatgagaaaataggggcctggagagtgatggacagagtcttgagtgtgaccctggacaactggacagtactcccatcctctctgggcctggatttgcccacctgggttgagggctgcccagagacctggcttctgttatctatgcaactggttgacctgtcttatcaggttgtgggtgcagatcagggcaggggtagggtggagttaatagaggcatttggactttagctgggaggagctgggagcgtcagacaatgaagtctacagaactgagcactcgagaccctgtggcttgggagctgggcctggccacagaggggcttgacgttgtcgaatgactgaacagactgagtcaaacacataacaaatgatgggataaatggtaaagtcagaaggggcaggccaggcgtggtggctcatgcctgtaatcctagcactttgggaggccgaggtgggcaaatcacctgaggtcaggagttcgagaccagcctggccaacatggtgaaaccccgtctctactaaaaatacaaaaattagccgggtgtggtggtgggcacctgtaatcccagctacttgggaggctgaggcaggataatcgcctgaacccagaaggcagaggttgcagtgagccaagattgcaccactgcactccagcctgggtgtcagtgctctgtctcaaaaagaaagagagagagagagagaaagaaagaaaaagaaaaaaagaaagaaagagaaaagaaaagagaaaaagaaacaggctgatgaatatcccctctgtagctagcccgagttaaacagtgatcctttctggggagtcagggagcgcttcatggaggaagaacaatgtggatgggccatgaaggatgagtaggagtttgccaagtggaaaagacttctggaagcggtttccagaaggaagaaacagcctgagcaagggcctggcacagggtgagagcagtttcagggaacagcattgatggatgaacagacactttagtctcttcccctggggcttccaggagtctgccccttcccccaccagggagagtggggcgatgcctcagcactgggcctggcctccctgacttggcttccctctccacagccccctgtgggtggcattgatgagcgccctaatcctgggtctgcttttcgtggcggtctacagcttgtcccatggcgaggtctcctatgacccactctatgctggtgagtcagtgggaagctgtggggaagaagactgtccaggcaagggcctccaccctcagacttgggggccattaaggggcctcctccatcagactgggggccctttaagagctcccatcagactggagacctcaaagagatttgaacactcccattaaactggggaacctcaaagagcctcccccttcagagctggggctcctaagaacagggactgcatctcctgcatcagattagaagctcctgaaaaagagtatactgcctcatcactttgagatctcctgagggcagggacggtgcctctcccatgagactggggactcccaaaggcaggcactgggcctctgaatcaaaccagggacttctgagagccaggctgtgtctcctccatcagacatgcagaatgaggcaggactgtggtcatgcaacctttggggttggggcagggactgggcctggagtccttgcctggaataatctcatccctgaccttaacttcaagccccgcccacactaagccctagccccacccacacgtgtcccctcccacacctgacccggcccgcccactcactgcagtcttcgctgtcttcgccttcacctcggttgtggacctcatcatcgctcttcaggaagacagctatgtggtgggcttcatggagttctacaccaaggaggtacttgggggacgaccagggagccccctaccgcactgcccgtctgagtctcccacctgcccccacagggagagccatacctgcgcacagcgcacggagtcttcatctgctactgggatggcactgttcactacctcctctacctggccatggccggcgccatctgcagaaggtgcaggaggcagggagagggtggcccctgaccctgggagagaagttgcatcctcagatggggtcccagggcagggtggagccagaagtgtctgtaggagaaatcaggacgcctctctagggctccagccaggggtggccaggagaaggttccagggaacgtctcaggtgtaggtggtggcctagcattgcttacatccaccctgtgcctgggcagccacttctgttcttggacagagggtctcactgttatttccccgttcaactccctgttgtcccttccatcctgggcaaaactgaaagggacccggagctgggaaacccacggtggtctccaggccctggctggggctctgagattacggagtgactacctgctggtcacccctccatcccctgctcaggaagagataccggaattttggactctactggctgggttccttcgccatgagcatcctggtgttccttacaggaaacattcttggtaaggacaaggctttgggaaatccaggttctcttgggcttggtcactgccctgcacctagaagcacccccattggatcctccatcccttccctgatgtctgcagaggccccacctccctctttgcgtgtccacagcctcagtcagcagcccacccctttccggtccctgtttcctcttggaaggcgggagaacccaactctgcttcctccccaggcaatggttcccagccccaggggtttgacccagaatggtcttgacacaggaagggaattttagggtgaatcttggggacagggtgaaagcttcaggggtaggtcttgggaggtagagcagtgaaggcagtctgggaggttggcatggcaaaacctcagcaaagggaacactcaaggtgtatttgtaggaagcaaagaacccactggaaggtaggatccatattcagaaggtaaattgaggcaggctaggctaaggagtatggacatcatcctgtgggcactagggagccatggaaggtggtggagcttgaatgaggatggtatttctgaatcaagatgtccagccagagaggccacgtgtggtggctcatgcctgtaatccttatgttgctcaggctggtctccaactctcggctcaagcaatccacctgcctcatcaatcacttgagccgtggagatcaagatcagcctgggcagcatggtgaaaccctgcctatactaaaagtacaaaaattagccaggtataatcccagctactcaggaggctgagacaagagaattgcttgaacctgggaggcagaggttgcagtgagccaagattgcatcactgcactccagcctgggtgacagagcaagactctgtctcagaacaaacaaacaaacagatgtccagcagggttctggcatggctgatgccctctctcctgcaccatggaaggcaaatacagctccgagatcaggcctgccttcttcctcaccatcccctacctgctggtgccatgctgggctggcatgaaggtcttcagccagccccgggcgctaacccgctgcaccgccaacatggtgagtgccttacccctcttaggccttgtcccaatgtgcctgaactttccccgtgtcagttgcttttggtcaaagacttaatttctgtggaaggttctcctttgtcacaagaaagaagggagggctgggtgcggtggctcatgcctgtaatcccaacattttgggaggccaaggcatgaggatcgcttgagcccaggaattggagaccagcctgggcaacacagccagattttttaactctacaaaaagttaaaaaattagccagatgtggtggtgcatgcctgtggtcccagctattcgggaggctgaggtgggaggatcacttgagcccaggagattaaggctgcagtgagctgagactgtgctgcttcactcaagcctgggcaacagaatgagaccctgtctcaaaaaaaaaaaaaaagaaaaaagaaaaaaaagaaaaaaagaaagaagggaggagccttaggaacctttattgagtacctactgaatacttgtcattgactacctctcatgctgtctgtttctctcccctgggccaggtgcaagaggaacaaagaaagggactcctgcagcgtccggctgacctggcccttgtcatatatctcatccttgctggcttcttcactctgttccggggcctggtgagtctgcgctggttggtctccccctcccctgccaccagtctcccttccctgacccacctctcccacactgcccttcctgtttgatcatccaaggaagttcttcatcaagtctaacctgagtgttccatgacaaagccccatttctcccagccagcccaacttgagctgggctgggagaggccagagcaaggggtgtgggcctgggagggtgggggaggcttcctgtgggaggtatgtctgagggttcttggtatgtctgtctgctccaggtggtgcttgattgccccacagatgcctgctttgtctatatctaccagtatgagccatacctgcgggaccctgtggcctaccctaaggtgcaggtgagaggggagcggggagaagaccacacccctgccatgggtaggggtccactgggcctctttgaagcaggtgccagaagcacaactcaaacaggcagaagcccatatggaatttactgtcctaccaaaaaaggacagatgtggtcttcaggtatggctggatccaggtgctcaaggtgcagactctgggctcttcttttcttttcttttcctttcttttctttctttctttttcttttttttttttttttttaaacagagttttgctcttgtggcccaggctggagtgcaatggcatgatctcggctcactgcaacctccacctcctgggctcaagtgattctcctgcctcagcctcccaagtagctgggattacaggcgtgagccaccatactcagctaattttgtatttttagtagatacggggttttgccatgttggtcaggctggtctcgaactcctgacctcaagtgatccacccacctcggcctcccaaagtgctgggattacaggcatgagccaccatgcccggcctctgagctctgctttctttgcatggcttcactctcaggcagtccctttatggggtggcagagacagcctgtggcagcttcaggcttccatgcaccccactcagccaccccagagcaatgtgagcccttattacccccgagcttaagcacaagtcttaggcaggctcagattggcccagcgtgaatcacttgcccatcccttactgagcatcatggacagggggctggaatgctccgactggctaggccagggtcgcatgccactttcagagaaaggttagtaggtttggtgtatgtgttcgggggttgggggcaaggatccccaagggaaatagaggagcactttgcagagagcctgggtggggtctgaggccatccagatccttcctcagggcctccacctcaggggtctcaggagacccacctggggtagctgctcatctcacaggctggtgcccctctcctcccgcccctgcagatgctgatgtacatgttttatgtcctgcctttctgcggcctggctgcctatgctctcaccttccctggttgctcctggcttccagactgggccttggtgtttgctggaggcatcggccaggtgaggtggcggatgggtgggtgagcaggcatgtgggagggaatttctgtctactcatcaatgcctttggtgtcctccctgggcactgtaatgatgagcccccaagaggccccagccccaggcccaatatcccaggattccctagtctaggggagacaaagccagatacagacactccaagccccatgaaaatagggacaggggctgtgaaggattccagaggggaaaggtttcctagaagcaaggcataggagctaggctttgatgtacgaggatgagttctccaggcagggaagggcattccaggaatgggaacagcacaaggagaagcacagagggagagagtgacttagcagggccataacccaggtaaaggcagataagagaaattggcagctggatgctgaaggctttgaactctgggactaggggcttgtactgagggtgatggggcgtttgaggaggagtttgagcagtgaggggcccagtcagagctaggagcctttttctgggttcctgatgaaaagtgctaaatcctgggccccggccagggaagtagggaccaggaaaacatttagaatccacaggatttgtgccaagacctctggggtggggaagactgggaggaggatctggagccaggtcagagagagatggggtgcagggcccaggagatggggttaggcaagttgggggggactcacagacaagtggacaagcacagggagggacagacaggacatgtaagggcaggaatctttacagacagaaggccaggtgaggtggctcacacctgtaatcccagcattttgggaggccgaggtgggagggctgcttgagcccaggagtctgagaccagcctaggcaacatggcaaaaacctgtctctacaaaaagtacaaaaattagctgggcatggtagcacgtgcctgctgtgctagctactcgggaggctgagattggaggatcacttgagcccaggaggttggggctgcagtgagccatgattgtgccactgcactccagcctggccaacagagcaagaccctatctctaaatagatagatagatagatggatggatggatagatagatagatagatagatagatagatagatagatagatagaaattttaaaaataggccaggcatggtggcttatgcctgtaatcctagcactttgggaggccaagatggatggattgcctgacctcaggagttcgagaccagcctgggcaacatgatgataccccatctctactaaaaatacaaaaaattaactgggcatagaggtgcacgcctgtagtcccagctactcagaggaggctgaagcacgagaatcacttgaacccaggaggcagcggaggttgcagtgaaccgagattgcaccactgcactccagcatgggcaacagaatgagactgtgtctcaaaaaaaaaaaaaaaaaaaaacagatagatggactggagatgggaaacagatagatgagcaaagcccgagaggtggggatgggcatcccctgggttctgcctgacctacctggggggctgtcggtgatgctgggatttcagttccttcctggcccctgacatccatcttccctgtctggctaccaggcacagttctcgcacatgggggcttccatgcacctgcgcacacccttcacctaccgtgtgcctgaggacacctggggctgcttcttcgtgtgcaatctgctgtatgcgctgggcccccacctgctggcctaccgttgccttcagtggcccgcattcttccaccagccaccaccctccgaccccctagccctccacaagaagcagcattgagagagctgtggactcaggacccaggactctgtttacgtgcccagtcagccctacctggggaagcgggggttgggtgttttagagacaggagggacatctccgggtgtctttagtcttggctatggtagtttcagtccagtgggtgggatggagaccaacgaccaagtgttcctgcaaggagagcctcccacagctgtcaccatgctccaactcccacacaaacgcttctaccccttccagaacttacccatcatccccccatggatcctttcagtaaaaaccctttcaatttccaaaat

SEQ ID NO: 2 - DNA, 10901 bp, Homo sapiens
attttggaaattgaaagggtttttactgaaaggatccatggggggatgatgggtaagttctggaaggggtagaagcgtttgtgtgggagttggagcatggtgacagctgtgggaggctctccttgcaggaacacttggtcgttggtctccatcccacccactggactgaaactaccatagccaagactaaagacacccggagatgtccctcctgtctctaaaacacccaacccccgcttccccaggtagggctgactgggcacgtaaacagagtcctgggtcctgagtccacagctctctcaatgctgcttcttgtggagggctagggggtcggagggtggtggctggtggaagaatgcgggccactgaaggcaacggtaggccagcaggtgggggcccagcgcatacagcagattgcacacgaagaagcagccccaggtgtcctcaggcacacggtaggtgaagggtgtgcgcaggtgcatggaagcccccatgtgcgagaactgtgcctggtagccagacagggaagatggatgtcaggggccaggaaggaactgaaatcccagcatcaccgacagccccccaggtaggtcaggcagaacccaggggatgcccatccccacctctcgggctttgctcatctatctgtttcccatctccagtccatctatctgtttttttttttttttttttttgagacacagtctcattctgttgcccatgctggagtgcagtggtgcaatctcggttcactgcaacctccgctgcctcctgggttcaagtgattctcgtgcttcagcctcctctgagtagctgggactacaggcgtgcacctctatgcccagttaattttttgtatttttagtagagatggggtatcatcatgttgcccaggctggtctcgaactcctgaggtcaggcaatccatccatcttggcctcccaaagtgctaggattacaggcataagccaccatgcctggcctatttttaaaatttctatctatctatctatctatctatctatctatctatctatctatccatccatccatctatctatctatctatttagagatagggtcttgctctgttggccaggctggagtgcagtggcacaatcatggctcactgcagccccaacctcctgggctcaagtgatcctccaatctcagcctcccgagtagctagcacagcaggcacgtgctaccatgcccagctaatttttgtactttttgtagagacaggtttttgccatgttgcctaggctggtctcagactcctgggctcaagcagccctcccacctcggcctcccaaaatgctgggattacaggtgtgagccacctcacctggccttctgtctgtaaagattcctgcccttacatgtcctgtctgtccctccctgtgcttgtccacttgtctgtgagtcccccccaacttgcctaaccccatctcctgggccctgcaccccatctctctctgacctggctccagatcctcctcccagtcttccccaccccagaggtcttggcacaaatcctgtggattctaaatgttttcctggtccctacttccctggccggggcccaggatttagcacttttcatcaggaacccagaaaaaggctcctagctctgactgggcccctcactgctcaaactcctcctcaaacgccccatcaccctcagtacaagcccctagtcccagagttcaaagccttcagcatccagctgccaatttctcttatctgcctttacctgggttatggccctgctaagtcactctctccctctgtgcttctccttgtgctgttcccattcctggaatgcccttccctgcctggagaactcatcctcgtacatcaaagcctagctcctatgccttgcttctaggaaacctttcccctctggaatccttcacagcccctgtccctattttcatggggcttggagtgtctgtatctggctttgtctcccctagactagggaatcctgggatattgggcctggggctggggcctcttgggggctcatcattacagtgcccagggaggacaccaaaggcattgatgagtagacagaaattccctcccacatgcctgctcacccacccatccgccacctcacctggccgatgcctccagcaaacaccaaggcccagtctggaagccaggagcaaccagggaaggtgagagcataggcagccaggccgcagaaaggcaggacataaaacatgtacatcagcatctgcaggggcgggaggagaggggcaccagcctgtgagatgagcagctaccccaggtgggtctcctgagacccctgaggtggaggccctgaggaaggatctggatggcctcagaccccacccaggctctctgcaaagtgctcctctatttcccttggggatccttgcccccaacccccgaacacatacaccaaacctactaacctttctctgaaagtggcatgcgaccctggcctagccagtcggagcattccagccccctgtccatgatgctcagtaagggatgggcaagtgattcacgctgggccaatctgagcctgcctaagacttgtgcttaagctcgggggtaataagggctcacattgctctggggtggctgagtggggtgcatggaagcctgaagctgccacaggctgtctctgccaccccataaagggactgcctgagagtgaagccatgcaaagaaagcagagctcagaggccgggcatggtggctcatgcctgtaatcccagcactttgggaggccgaggtgggtggatcacttgaggtcaggagttcgagaccagcctgaccaacatggcaaaaccccgtatctactaaaaatacaaaattagctgagtatggtggctcacgcctgtaatcccagctacttgggaggctgaggcaggagaatcacttgagcccaggaggtggaggttgcagtgagccgagatcatgccattgcactccagcctgggccacaagagcaaaactctgtttaaaaaaaaaaaaaaaaaagaaaaagaaagaaagaaaagaaaggaaaagaaaagaaaagaagagcccagagtctgcaccttgagcacctggatccagccatacctgaagaccacatctgtccttttttggtaggacagtaaattccatatgggcttctgcctgtttgagttgtgcttctggcacctgcttcaaagaggcccagtggacccctacccatggcaggggtgtggtcttctccccgctcccctctcacctgcaccttagggtaggccacagggtcccgcaggtatggctcatactggtagatatagacaaagcaggcatctgtggggcaatcaagcaccacctggagcagacagacataccaagaaccctcagacatacctcccacaggaagcctcccccaccctcccaggcccacaccccttgctctggcctctcccagcccagctcaagttgggctggctgggagaaatggggctttgtcatggaacactcaggttagacttgatgaagaacttccttggatgatcaaacaggaagggcagtgtgggagaggtgggtcagggaagggagactggtggcaggggagggggagaccaaccagcgcagactcaccaggccccggaacagagtgaagaagccagcaaggatgagatatatgacaagggccaggtcagccggacgctgcaggagtccctttctttgttcctcttgcacctggcccaggggagagaaacagacagcatgagaggtagtcaatgacaagtattcagtaggtactcaataaaggttcctaaggctcctcccttctttctttttttcttttttttcttttttctttttttttttttttgagacagggtctcattctgttgcccaggcttgagtgaagcagcacagtctcagctcactgcagccttaatctcctgggctcaagtgatcctcccacctcagcctcccgaatagctgggaccacaggcatgcaccaccacatctggctaattttttaactttttgtagagttaaaaaatctggctgtgttgcccaggctggtctccaattcctgggctcaagcgatcctcatgccttggcctcccaaaatgttgggattacaggcatgagccaccgcacccagccctcccttctttcttgtgacaaaggagaaccttccacagaaattaagtctttgaccaaaagcaactgacacggggaaagttcaggcacattgggacaaggcctaagaggggtaaggcactcaccatgttggcggtgcagcgggttagcgcccggggctggctgaagaccttcatgccagcccagcatggcaccagcaggtaggggatggtgaggaagaaggcaggcctgatctcggagctgtatttgccttccatggtgcaggagagagggcatcagccatgccagaaccctgctggacatctgtttgtttgtttgttctgagacagagtcttgctctgtcacccaggctggagtgcagtgatgcaatcttggctcactgcaacctctgcctcccaggttcaagcaattctcttgtctcagcctcctgagtagctgggattatacctggctaatttttgtacttttagtataggcagggtttcaccatgctgcccaggctgatcttgatctccacggctcaagtgattgatgaggcaggtggattgcttgagccgagagttggagaccagcctgagcaacataaggattacaggcatgagccaccacacgtggcctctctggctggacatcttgattcagaaataccatcctcattcaagctccaccaccttccatggctccctagtgcccacaggatgatgtccatactccttagcctagcctgcctcaatttaccttctgaatatggatcctaccttccagtgggttctttgcttcctacaaatacaccttgagtgttccctttgctgaggttttgccatgccaacctcccagactgccttcactgctctacctcccaagacctacccctgaagctttcaccctgtccccaagattcaccctaaaattcccttcctgtgtcaagaccattctgggtcaaacccctggggctgggaaccattgcctggggaggaagcagagttgggttctcccgccttccaagaggaaacagggaccggaaaggggtgggctgctgactgaggctgtggacacgcaaagagggaggtggggcctctgcagacatcagggaagggatggaggatccaatgggggtgcttctaggtgcagggcagtgaccaagcccaagagaacctggatttcccaaagccttgtccttaccaagaatgtttcctgtaaggaacaccaggatgctcatggcgaaggaacccagccagtagagtccaaaattccggtatctcttcctgagcaggggatggaggggtgaccagcaggtagtcactccgtaatctcagagccccagccagggcctggagaccaccgtgggtttcccagctccgggtccctttcagttttgcccaggatggaagggacaacagggagttgaacggggaaataacagtgagaccctctgtccaagaacagaagtggctgcccaggcacagggtggatgtaagcaatgctaggccaccacctacacctgagacgttccctggaaccttctcctggccacccctggctggagccctagagaggcgtcctgatttctcctacagacacttctggctccaccctgccctgggaccccatctgaggatgcaacttctctcccagggtcaggggccaccctctccctgcctcctgcaccttctgcagatggcgccggccatggccaggtagaggaggtagtgaacagtgccatcccagtagcagatgaagactccgtgcgctgtgcgcaggtatggctctccctgtgggggcaggtgggagactcagacgggcagtgcggtagggggctccctggtcgtcccccaagtacctccttggtgtagaactccatgaagcccaccacatagctgtcttcctgaagagcgatgatgaggtccacaaccgaggtgaaggcgaagacagcgaagactgcagtgagtgggcgggccgggtcaggtgtgggaggggacacgtgtgggtggggctagggcttagtgtgggcggggcttgaagttaaggtcagggatgagattattccaggcaaggactccaggcccagtccctgccccaaccccaaaggttgcatgaccacagtcctgcctcattctgcatgtctgatggaggagacacagcctggctctcagaagtccctggtttgattcagaggcccagtgcctgcctttgggagtccccagtctcatgggagaggcaccgtccctgccctcaggagatctcaaagtgatgaggcagtatactctttttcaggagcttctaatctgatgcaggagatgcagtccctgttcttaggagccccagctctgaagggggaggctctttgaggttccccagtttaatgggagtgttcaaatctctttgaggtctccagtctgatgggagctcttaaagggcccccagtctgatggaggaggccccttaatggcccccaagtctgagggtggaggcccttgcctggacagtcttcttccccacagcttcccactgactcaccagcatagagtgggtcataggagacctcgccatgggacaagctgtagaccgccacgaaaagcagacccaggattagggcgctcatcaatgccacccacagggggctgtggagagggaagccaagtcagggaggccaggcccagtgctgaggcatcgccccactctccctggtgggggaaggggcagactcctggaagccccaggggaagagactaaagtgtctgttcatccatcaatgctgttccctgaaactgctctcaccctgtgccaggcccttgctcaggctgtttcttccttctggaaaccgcttccagaagtcttttccacttggcaaactcctactcatccttcatggcccatccacattgttcttcctccatgaagcgctccctgactccccagaaaggatcactgtttaactcgggctagctacagaggggatattcatcagcctgtttctttttctcttttcttttctctttctttctttttttctttttctttctttctctctctctctctctttctttttgagacagagcactgacacccaggctggagtgcagtggtgcaatcttggctcactgcaacctctgccttctgggttcaggcgattatcctgcctcagcctcccaagtagctgggattacaggtgcccaccaccacacccggctaatttttgtatttttagtagagacggggtttcaccatgttggccaggctggtctcgaactcctgacctcaggtgatttgcccacctcggcctcccaaagtgctaggattacaggcatgagccaccacgcctggcctgccccttctgactttaccatttatcccatcatttgttatgtgtttgactcagtctgttcagtcattcgacaacgtcaagcccctctgtggccaggcccagctcccaagccacagggtctcgagtgctcagttctgtagacttcattgtctgacgctcccagctcctcccagctaaagtccaaatgcctctattaactccaccctacccctgccctgatctgcacccacaacctgataagacaggtcaaccagttgcatagataacagaagccaggtctctgggcagccctcaacccaggtgggcaaatccaggcccagagaggatgggagtactgtccagttgtccagggtcacactcaagactctgtccatcactctccaggcccctattttctcatgatcccctcagaacccaagatttccatcctgaccccatctaacaatgacattatagtactcagatgagaccaagacaaatctttgtacacagtttataatccttaaccgtaactatgagatgagatctaggatcgtgcccattacactgatgagggaactgaggctcccagaggaacttggctcacccaggatcccaggagatggagatgggtattcccacccagggagccaggctcatggttaagactctctccaccccatggcttgggttgagctgggtttagaagtacgaggggcttgcagatgcccactatccggtggctggacccacagggctaggatctagggttaggagacagggaccaggaaagggaaccagtagggggaactgagtctagggacatggttagccagccctgaacaagaggaaagtcacaggcctgagacaggcaatggagtagggtgtgtgtgtgtgtgtgtgtgtgtgtgtgtgtgtgtgagcaggagtcaggtacccggggccttatctgggacaatacttttacccttggtgactttggaacctaggcagggcgcatccctgggaaaaccccagaaaccctccaaagctctggcttgtggggactcatcattccttcttcccaggccacaaacatcccaggagcggccgcatcccagcctccagcccggcgggaaggggacttccggttagaggggggtgttcttctggcccaccccaatcctgccgggtcggagctgagctggggcgcagggctcgcagaagccaggtccgcggaccgcgcatcctccctccagcccacctccagtcctccccgcccccgcccgcccccactgtccccaaggccgccctggcccctctccgcacgcactgcgagagcgccgagacgtggttgagcgcgtaggacaccgggagggcgctcagcgacagcgccgcgatcttgccggccagcggcgggatgtccatagcggcggctgctggaccccggctcagccccgacgcgttctccagggcgctcggctcctcgttggcggcgagtccgggccgaggctgccagggacccgccccgcacaaaggtcgaccccgctgcgccctgggcaggccgccgtgaccgccctgcgtgttcccagggagcctccaaggcccctccccggccctccccctggcagctgccccgccccttcgcccctcaccatcgacaccctcgtctccaatggccgtcccgctactcagcctcagtttccctcactgtcaaaggctgggacacaacacctcgggatgcttctgctcttaggccaaggggtgcgccctggaggtcctggcgtgccccctctttcccctgcctccacaacttcgttctaaggaaattttctcctggactctgcgcttctaaacctctgcattccccagagtttcccatccccacccaaagatcaagtcggcattccctgtgcgcacggatggagcaacctccagctcttgggtgcaaaatgcctttcagtgggcttagatttgagttttcataaggtggccacaaatgtaaacgtgtttccaggcaggtgtgaagtttttttgtttgttttttgagaggtctcactctgtggcccagactggagtgcagtggccctcctccttgaactcccagcctcaagagatcctcctacctcagcctcccaagtagttgggactacaggtatgcaccaccacgcgcagctagttattttttgtaaagacagaggtctcacttttttgcccagactggtttcaaactcctgggctcaacagatcctcccacatcagcctcccgaggagctgggattacaggcgtgagccactgcgaggggtctttaagtgtgaggctttgactccggggctgtccctttgcaggctagtcccgggtttagggttcttcatttcggggagagggtagaaggggtcctagcgggtgggggctgaagttagaatatcgggatggagccagtttggtgaagagtttgggaacggtgttcctggcagggaggaaagtggctcaggcttggaactgagcagtggaaaggaggtcggttctgctggggtgtgatgagaagcgagacagctgtgagaggctgtgggaggttttgaacagctgggagggggccacagtattgggggggagaataaggagaccatctgtctttgtcaccccctccaaccagactctggcccatgtggagtacttgtggatgctgcagacagcaaggtgaaccatgcccacctgacgcctgccctgcgggaccccagtctgcagctggcacaaattctaaccactgcccctacctcaggccccattctgcacgcagccccttagcttgatgccaactgggtcacaggtcttcctgaactgggccacaagagggtcttctggccgcaggtctgactcagcctccttccccaggtgtccactgcccatgggtgaagttcaggttcccctggactttccccaactctagcagggtcaacaccccccaggcctgctttctgtctgtaaaatgagccttcttgtaagcgggccccagcatcccctcctccaggcagccctgcctgccacccccaccccaccttctccacacaaggccagggtgcctgtgcccagctcagcctaggggcttggccttgtcccgtgtacaggatgcacctgcacacgcacacagcacttggaggcctcgtcccctggcaaggggtaaagtccatgccctgagcctggtgagcctccaggttgctgagaactgagaagtgacttggatggctgaatgcctgggacccagtgccaggattccctgaaccactggctgcagagaactaccccgctgtgctcagggtcctggcccactgccttctgggcagccctcattcatgggcacccaggccaagcccaccaatgttactctttgctctgcctcagccacagcgtcaggaaagaacaaagggtggtatatcaccccagccttggctctgccactgcatctggcacctccct

SEQ ID NO: 3 - RNA, 1483 nt, Homo sapiens
gcgcccuggagaacgcgucggggcugagccgggguccagcagccgccgcuauggacaucccgccgcuggccggcaagaucgcggcgcugucgcugagcgcccucccgguguccuacgcgcucaaccacgucucggcgcucucgcacccccuguggguggcauugaugagcgcccuaauccugggucugcuuuucguggcggucuacagcuugucccauggcgaggucuccuaugacccacucuaugcugucuucgcugucuucgccuucaccucgguuguggaccucaucaucgcucuucaggaagacagcuauguggugggcuucauggaguucuacaccaaggagggagagccauaccugcgcacagcgcacggagucuucaucugcuacugggauggcacuguucacuaccuccucuaccuggccauggccggcgccaucugcagaaggaagagauaccggaauuuuggacucuacuggcuggguuccuucgccaugagcauccugguguuccuuacaggaaacauucuuggcaaauacagcuccgagaucaggccugccuucuuccucaccauccccuaccugcuggugccaugcugggcuggcaugaaggucuucagccagccccgggcgcuaacccgcugcaccgccaacauggugcaagaggaacaaagaaagggacuccugcagcguccggcugaccuggcccuugucauauaucucauccuugcuggcuucuucacucuguuccggggccugguggugcuugauugccccacagaugccugcuuugucuauaucuaccaguaugagccauaccugcgggacccuguggccuacccuaaggugcagaugcugauguacauguuuuauguccugccuuucugcggccuggcugccuaugcucucaccuucccugguugcuccuggcuuccagacugggccuugguguuugcuggaggcaucggccaggcacaguucucgcacaugggggcuuccaugcaccugcgcacacccuucaccuaccgugugccugaggacaccuggggcugcuucuucgugugcaaucugcuguaugcgcugggcccccaccugcuggccuaccguugccuucaguggcccgcauucuuccaccagccaccacccuccgacccccuagcccuccacaagaagcagcauugagagagcuguggacucaggacccaggacucuguuuacgugcccagucagcccuaccuggggaagcggggguuggguguuuuagagacaggagggacaucuccgggugucuuuagucuuggcuaugguaguuucaguccagugggugggauggagaccaacgaccaaguguuccugcaaggagagccucccacagcugucaccaugcuccaacucccacacaaacgcuucuaccccuuccagaacuuacccaucauccccccauggauccuuucaguaaaaacccuuucaauuuccaaaau

SEQ ID NO: 4 - RNA, 1483 nt, Homo sapiens
auuuuggaaauugaaaggguuuuuacugaaaggauccauggggggaugauggguaaguucuggaagggguagaagcguuugugugggaguuggagcauggugacagcugugggaggcucuccuugcaggaacacuuggucguuggucuccaucccacccacuggacugaaacuaccauagccaagacuaaagacacccggagaugucccuccugucucuaaaacacccaacccccgcuuccccagguagggcugacugggcacguaaacagaguccuggguccugaguccacagcucucucaaugcugcuucuuguggagggcuagggggucggagggugguggcugguggaagaaugcgggccacugaaggcaacgguaggccagcaggugggggcccagcgcauacagcagauugcacacgaagaagcagccccagguguccucaggcacacgguaggugaagggugugcgcaggugcauggaagcccccaugugcgagaacugugccuggccgaugccuccagcaaacaccaaggcccagucuggaagccaggagcaaccagggaaggugagagcauaggcagccaggccgcagaaaggcaggacauaaaacauguacaucagcaucugcaccuuaggguaggccacagggucccgcagguauggcucauacugguagauauagacaaagcaggcaucuguggggcaaucaagcaccaccaggccccggaacagagugaagaagccagcaaggaugagauauaugacaagggccaggucagccggacgcugcaggagucccuuucuuuguuccucuugcaccauguuggcggugcagcggguuagcgcccggggcuggcugaagaccuucaugccagcccagcauggcaccagcagguaggggauggugaggaagaaggcaggccugaucucggagcuguauuugccaagaauguuuccuguaaggaacaccaggaugcucauggcgaaggaacccagccaguagaguccaaaauuccgguaucucuuccuucugcagauggcgccggccauggccagguagaggagguagugaacagugccaucccaguagcagaugaagacuccgugcgcugugcgcagguauggcucucccuccuugguguagaacuccaugaagcccaccacauagcugucuuccugaagagcgaugaugagguccacaaccgaggugaaggcgaagacagcgaagacagcauagagugggucauaggagaccucgccaugggacaagcuguagaccgccacgaaaagcagacccaggauuagggcgcucaucaaugccacccacagggggugcgagagcgccgagacgugguugagcgcguaggacaccgggagggcgcucagcgacagcgccgcgaucuugccggccagcggcgggauguccauagcggcggcugcuggaccccggcucagccccgacgcguucuccagggcgc

SEQ ID NO: 5 - RNA, 21 nt, Artificial Sequence
  siRNA
ccucgguuguggaccucauuu

SEQ ID NO: 6 - RNA, 19 nt, Artificial Sequence
  siRNA
ggaagagauaccggaauuu

SEQ ID NO: 7 - RNA, 19 nt, Artificial Sequence
  siRNA
uagcgacuaaacacaucaa